European Patent Application EP 4 242 230 A1, published September 13, 2023. Title: ANTIBODY TARGETING INTERLEUKIN 36R,PREPARATION METHOD THEREFOR,AND APPLICATION THEREOF. Applicant: SHANGHAI HUAOTA BIOPHARMACEUTICAL CO., LTD. HUABO BIOPHARM (SHANGHAI) CO., LTD. The sequence listing filed with the application follows.

SEQUENCE LISTING (12 sequences)

SEQ ID NO: 1 - protein, 119 aa, Artificial Sequence
  VH
QVQLQQTGSVLVRPGTSVKLSCKASGYTFTSSWMHWAKQRPGQGLEWIGEIHPNSAKTNYNEKFKGKATLTVDTFSSTAYVDLSSLASEDSAVYYCARVDYGKPWFAYWGQGTLVTVSA

SEQ ID NO: 2 - protein, 108 aa, Artificial Sequence
  VL
QIVLTQSPTIMSASPGERVTMTCSASSSVSSSYLHWYQQKPGSSPKLWIYSTSNLASGVPARFSGSGSGTSYSLTINSMEAEDAATYYCQQFQSSPLTFGAGTKLGLK

SEQ ID NO: 3 - protein, 8 aa, Artificial Sequence
  CDR1
GYTFTSSW

SEQ ID NO: 4 - protein, 8 aa, Artificial Sequence
  CDR2
IHPNSAKT

SEQ ID NO: 5 - protein, 12 aa, Artificial Sequence
  CDR3
ARVDYGKPWFAY

SEQ ID NO: 6 - protein, 7 aa, Artificial Sequence
  CDR1’
SSVSSSY

SEQ ID NO: 7 - protein, 3 aa, Artificial Sequence
  CDR2’
STS

SEQ ID NO: 8 - protein, 9 aa, Artificial Sequence
  CDR3’
QQFQSSPLT

SEQ ID NO: 9 - protein, 119 aa, Artificial Sequence
  VH
QVQLVQSGAEVKKPGASVKVSCKASGYTFTSSWMHWAKQAPGQGLEWIGEIHPNSAKTNYNQKFQGRVTMTRDTSISTAYMELSRLRSDDTAVYYCARVDYGKPWFAYWGQGTLVTVSS

SEQ ID NO: 10 - protein, 108 aa, Artificial Sequence
  VL
EIVLTQSPGTLSLSPGERATLSCSASSSVSSSYLHWYQQKPGQAPRLWIYSTSNRATGIPDRFSGSGSGTDFTLTISRLEPEDFATYYCQQFQSSPLTFGQGTKLEIK

SEQ ID NO: 11 - protein, 108 aa, Artificial Sequence
  VL
QIVLTQSPGTLSLSPGERATLSCRASSSVSSSYLHWYQQKPGQAPRLWIYSTSSRATGIPDRFSGSGSGTDFTLTISRLEPEDFATYYCQQFQSSPLTFGQGTKLEIK

SEQ ID NO: 12 - protein, 108 aa, Artificial Sequence
  VL
QIVLTQSPGTLSLSPGERATLSCRASSSVSSSYLHWYQQKPGQAPRLLIYSTSSRATGIPDRFSGSGSGTDFTLTISRLEPEDFATYYCQQFQSSPLTFGQGTKLEIK